European Patent Specification EP 3 209 801 B1, published June 28, 2023. Title: Genome Methylation Analysis. Applicant: Commonwealth Scientific and Industrial Research Organisation. The sequence listing filed with the application follows.

SEQUENCE LISTING (3 sequences)

SEQ ID NO: 1 - DNA, 42 bp, Artificial Sequence
  Synthetic sequence
  modified_base (2)..(2): I
  modified_base (5)..(5): I
  modified_base (20)..(20): I
  modified_base (25)..(25): O-methylcytosine
  modified_base (26)..(26): O-methylthymine
  modified_base (27)..(27): O-methylcytosine
  modified_base (39)..(41): O-methylthymine
caccatccctctttctacaatgcgctctcttgcttttctttt

SEQ ID NO: 2 - DNA, 25 bp, Artificial Sequence
  Synthetic sequence
  modified_base (6)..(6): methylcytosine
  modified_base (8)..(9): methylcytosine
  modified_base (12)..(14): methylcytosine
  modified_base (16)..(16): methylcytosine
  modified_base (17)..(19): O-methylthymine
  modified_base (20)..(20): methylcytosine
  modified_base (23)..(23): methylcytosine
cccgtcgccgtccctctttctacag

SEQ ID NO: 3 - DNA, 17 bp, Artificial Sequence
  Synthetic sequence
tggggcggggtctagag